European Patent Specification EP 4 208 206 B1, published October 9, 2024. Title: Modified Cas9 System having a dominant negative effector on non-homologous end-joining  fused thereto and its use for improved gene editing. Applicant: Albert-Ludwigs-Univ. Freiburg. The sequence listing filed with the application follows.

SEQUENCE LISTING (2 sequences)

SEQ ID NO: 1 - protein, 498 aa, artificial sequence
  dn53BP1
GEEEFDMPQPPHGHVLHRHMRTIREVRTLVTRVITDVYYVDGTEVERKVTEETEEPIVECQECETEVSPSQTGGSSGDLGDISSFSSKASSLHRTSSGTSLSAMHSSGSSGKGAGPLRGKTSGTEPADFALPSSRGGPGKLSPRKGVSQTGTPVCEEDGDAGLGIRQGGKAPVTPRGRGRRGRPPSRTTGTRETAVPGPLGIEDISPNLSPDDKSFSRVVPRVPDSTRRTDVGAGALRRSDSPEIPFQAAAGPSDGLDASSPGNSFVGLRVVAKWSSNGYFYSGKITRDVGAGKYKLLFDDGYECDVLGKDILLCDPIPLDTEVTALSEDEYFSAGVVKGHRKESGELYYSIEKEGQRKWYKRMAVILSLEQGNRLREQYGLGPYEAVTPLTKAADISLDNLVEGKRKRRSNVSSPATPTASSSSSTTPTRKITESPRASMGVLSGKRKLITSEEERSPAKRGRKSATVKPGAVGAGEFVSPCESGDNTGEPSALEEQ

SEQ ID NO: 2 - protein, 527 aa, artificial sequence
  RNF 168 DRING
MALPKDAIPSLSECSSWTRYHTRRNSLVNVELWTIIQKHYPRECKLRASGQESEEVADDYQPVRLLSKPGELRREYEEEISKVAAERRASEEEENKASEEYIQRLLAEEEEEEKRQAEKRRRAMEEQLKSDEELARKLSIDINNFCEGSISASPLNSRKSDPVTPKSEKKSKNKQRNTGDIQKYLTPKSQFGSASHSEAVQEVRKDSVSKDIDSSDRKSPTGQDTEIEDMPTLSPQISLGVGEQGADSSIESPMPWLCACGAEWYHEGNVKTRPSNHGKELCVLSHERPKTRVPYSKETAVMPCGRTESGCAPTSGVTQTNGNNTGETENEESCLLISKEISKRKNQESSFEAVKDPCFSAKRRKVSPESSPDQEETEINFTQKLIDLEHLLFERHKQEEQDRLLALQLQKEVDKEQMVPNRQKGSPDEYHLRATSSPPDKVLNGQRKNPKDGNFKRQTHTKHPTPERGSRDKNRQVSLKMQLKQSVNRRKMPNSTRDHCKVSKSAHSLQPSISQKSVFQMFQRCTK